European Patent Application EP 4 317 455 A1, published February 7, 2024. Title: Method and Composition for Amplifying Target Nucleic Acid using Guide Probe and Clamping probe. Applicant: PANAGENE INC. The sequence listing filed with the application follows.

SEQUENCE LISTING (9 sequences)

SEQ ID NO: 1 - DNA, 19 bp, Artificial Sequence
  partial primer 1
gcgtgactcgtctacgtca

SEQ ID NO: 2 - DNA, 29 bp, Artificial Sequence
  specific primer 1
gtgacatgttctaatatagtcacattttc

SEQ ID NO: 3 - DNA, 23 bp, Artificial Sequence
  guide probe 1
aaggcactcttgccgagtcacgc

SEQ ID NO: 4 - DNA, 15 bp, Artificial Sequence
  clamping probe 1
ctacgccaccagctc

SEQ ID NO: 5 - DNA, 14 bp, Artificial Sequence
  detection probe 1
taaacttgtggtag

SEQ ID NO: 6 - DNA, 19 bp, Artificial Sequence
  partial primer 2
gtcgtccgtgccttccaca

SEQ ID NO: 7 - DNA, 24 bp, Artificial Sequence
  specific primer 2
tgtagggcatttctgatgtgactc

SEQ ID NO: 8 - DNA, 25 bp, Artificial Sequence
  guide probe 2
agtgtcatcttgcctcacggacgac

SEQ ID NO: 9 - DNA, 13 bp, Artificial Sequence
  detection probe 2
cagcagtaaatct